European Patent Application EP 4 159 851 A1, published April 5, 2023. Title: DNA polymerase variants that show high discrimination against genetic variation. Applicant: Genotech Corporation. The sequence listing filed with the application follows.

SEQUENCE LISTING (100 sequences)

SEQ ID NO: 1 - protein, 832 aa, Thermus Aquaticus [sequence omitted]

SEQ ID NO: 2 - protein, 834 aa, Thermus sp.
MKAMLPLFEPKGRVLLVDGHHLAYRTFFALKGLTTSRGEPVQAVYGFAKSLLKALKEDGYKAVFVVFDAKAPSFRHEAYEAYKAGRAPTPEDFPRQLALIKELVDLLGFTRLEVPGFEADDVLATLAKKAEREGYEVRILTADRDLYQLVSDRVAVLHPEGHLITPEWLWEKYGLKPEQWVDFRALVGDPSDNLPGVKGIGEKTALKLLKEWGSLENILKNLDRVKPESVRERIKAHLEDLKLSLELSRVRSDLPLEVDFARRREPDREGLRAFLERLEFGSLLHEFGLLEAPAPLEEAPWPPPEGAFVGFVLSRPEPMWAELKALAACKEGRVHRAKDPLAGLKDLKEVRGLLAKDLAVLALREGLDLAPSDDPMLLAYLLDPSNTTPEGVARRYGGEWTEDAAHRALLAERLQQNLLERLKGEEKLLWLYQEVEKPLSRVLAHMEATGVRLDVAYLKALSLELAEEIRRLEEEVFRLAGHPFNLNSRDQLERVLFDELRLPALGKTQKTGKRSTSAAVLEALREAHPIVEKILQHRELTKLKNTYVDPLPGLVHPRTGRLHTRFNQTATATGRLSSSDPNLQNIPIRTPLGQRIRRAFVAEAGWALVALDYSQIELRVLAHLSGDENLIRVFQEGKDIHTQTASWMFGVSPEAVDPLMRRAAKTVNFGVLYGMSAHRLSQELAIPYEEAVAFIERYFQSFPKVRAWIEKTLEEGRKRGYVETLFGRRRYVPDLNARVKSVREAAERMAFNMPVQGTAADLMKLAMVKLFPHLREMGARMLLQVHDELLLEAPQARAEEVAALAKEAMEKAYPLAVPLEVEVGIGEDWLSAKG

SEQ ID NO: 3 - DNA, 501 bp, Homo Sapiens
aaaatattcgttttaagggtaaagaaaaaagttaaaaaatctatttacataaaaaataagaacactgatttttgtgaatactgggaactatgaaaatactatagttgagaccttcaatgactttctagtaactcagcagcatctcagggccaaaaatttaatcagtggaaaaatagcctcaattcttaccatccacaaaatggatccagacaactgttcaaactgatgggacccactccatcgagatttcactgtagctagaccaaaatcacctatttttactgtgaggtcttcatgaagaaatatatctgaggtgtagtaagtaaaggaaaacagtagatctcattttcctatcagagcaagcattatgaagagtttaggtaagagatctaatttctataattctgtaatataatattctttaaaacatagtacttcatctttcctcttagagtcaataagtatgtctaaaacaatgattagttctatttagcctatata

SEQ ID NO: 4 - DNA, 501 bp, Homo sapiens
aaaatattcgttttaagggtaaagaaaaaagttaaaaaatctatttacataaaaaataagaacactgatttttgtgaatactgggaactatgaaaatactatagttgagaccttcaatgactttctagtaactcagcagcatctcagggccaaaaatttaatcagtggaaaaatagcctcaattcttaccatccacaaaatggatccagacaactgttcaaactgatgggacccactccatcgagatttctctgtagctagaccaaaatcacctatttttactgtgaggtcttcatgaagaaatatatctgaggtgtagtaagtaaaggaaaacagtagatctcattttcctatcagagcaagcattatgaagagtttaggtaagagatctaatttctataattctgtaatataatattctttaaaacatagtacttcatctttcctcttagagtcaataagtatgtctaaaacaatgattagttctatttagcctatata

SEQ ID NO: 5 - DNA, 448 bp, Homo sapiens
cacgcacacacatatccccatggcaaactcttgctatcccaggagcgcagaccgcatgtgaggatcctggctccttatctcccctccccgtatctcccttccctgattacctttgcgatctgcacacaccagttgagcaggtactgggagccaatattgtctttgtgttcccggacatagtccaggaggcagccgaagggcatgagctgcgtgatgagctgcacggtggaggtgaggcagatgcccagcaggcggcacacgtgggggttgtccacgctggccatcacgtaggcttcctggagggagggagaggcacgtcagtgtggcttcgcatggtggccagaaggaggggcacatggaccccttccaggtgaagacgcatgaatgcgatcttgagtttcaaaatacgtactcatggaggaaaagctgtgcctgcaaaagacctagc

SEQ ID NO: 6 - DNA, 448 bp, Homo sapiens
cacgcacacacatatccccatggcaaactcttgctatcccaggagcgcagaccgcatgtgaggatcctggctccttatctcccctccccgtatctcccttccctgattacctttgcgatctgcacacaccagttgagcaggtactgggagccaatattgtctttgtgttcccggacatagtccaggaggcagccgaagggcatgagctgcatgatgagctgcacggtggaggtgaggcagatgcccagcaggcggcacacgtgggggttgtccacgctggccatcacgtaggcttcctggagggagggagaggcacgtcagtgtggcttcgcatggtggccagaaggaggggcacatggaccccttccaggtgaagacgcatgaatgcgatcttgagtttcaaaatacgtactcatggaggaaaagctgtgcctgcaaaagacctagc

SEQ ID NO: 7 - protein, 18 aa, Thermus Aquaticus
ELGLPAIGKTEKTGKRST

SEQ ID NO: 8 - DNA, 30 bp, Artificial Sequence
  primer
tttgacgagctaagacttcccgccatcggc

SEQ ID NO: 9 - DNA, 30 bp, Artificial Sequence
  primer
gccgatggcgggaagtcttagctcgtcaaa

SEQ ID NO: 10 - DNA, 30 bp, Artificial Sequence
  primer
cccgccatcggcgctacggagaagaccggc

SEQ ID NO: 11 - DNA, 30 bp, Artificial Sequence
  primer
gccggtcttctccgtagcgccgatggcggg

SEQ ID NO: 12 - DNA, 30 bp, Artificial Sequence
  primer
cccgccatcggcgaaacggagaagaccggc

SEQ ID NO: 13 - DNA, 30 bp, Artificial Sequence
  primer
gccggtcttctccgtttcgccgatggcggg

SEQ ID NO: 14 - DNA, 30 bp, Artificial Sequence
  primer
cccgccatcggctctacggagaagaccggc

SEQ ID NO: 15 - DNA, 30 bp, Artificial Sequence
  primer
gccggtcttctccgtagagccgatggcggg

SEQ ID NO: 16 - DNA, 30 bp, Artificial Sequence
  primer
cccgccatcggcggtacggagaagaccggc

SEQ ID NO: 17 - DNA, 30 bp, Artificial Sequence
  primer
gccggtcttctccgtaccgccgatggcggg

SEQ ID NO: 18 - DNA, 30 bp, Artificial Sequence
  primer
cccgccatcggcagaacggagaagaccggc

SEQ ID NO: 19 - DNA, 30 bp, Artificial Sequence
  primer
gccggtcttctccgttctgccgatggcggg

SEQ ID NO: 20 - DNA, 30 bp, Artificial Sequence
  primer
cccgccatcggcttcacggagaagaccggc

SEQ ID NO: 21 - DNA, 30 bp, Artificial Sequence
  primer
gccggtcttctccgtgaagccgatggcggg

SEQ ID NO: 22 - DNA, 30 bp, Artificial Sequence
  primer
cccgccatcggcattacggagaagaccggc

SEQ ID NO: 23 - DNA, 30 bp, Artificial Sequence
  primer
gccggtcttctccgtaatgccgatggcggg

SEQ ID NO: 24 - DNA, 30 bp, Artificial Sequence
  primer
cccgccatcggccttacggagaagaccggc

SEQ ID NO: 25 - DNA, 30 bp, Artificial Sequence
  primer
gccggtcttctccgtaaggccgatggcggg

SEQ ID NO: 26 - DNA, 30 bp, Artificial Sequence
  primer
cccgccatcggcatgacggagaagaccggc

SEQ ID NO: 27 - DNA, 30 bp, Artificial Sequence
  primer
gccggtcttctccgtcatgccgatggcggg

SEQ ID NO: 28 - DNA, 30 bp, Artificial Sequence
  primer
cccgccatcggctggacggagaagaccggc

SEQ ID NO: 29 - DNA, 30 bp, Artificial Sequence
  primer
gccggtcttctccgtccagccgatggcggg

SEQ ID NO: 30 - DNA, 30 bp, Artificial Sequence
  primer
atcggcaagacggctaagaccggcaagcgc

SEQ ID NO: 31 - DNA, 30 bp, Artificial Sequence
  primer
gcgcttgccggtcttagccgtcttgccgat

SEQ ID NO: 32 - DNA, 30 bp, Artificial Sequence
  primer
atcggcaagacgaagaagaccggcaagcgc

SEQ ID NO: 33 - DNA, 30 bp, Artificial Sequence
  primer
gcgcttgccggtcttcttcgtcttgccgat

SEQ ID NO: 34 - DNA, 30 bp, Artificial Sequence
  primer
atcggcaagacgtctaagaccggcaagcgc

SEQ ID NO: 35 - DNA, 30 bp, Artificial Sequence
  primer
gcgcttgccggtcttagacgtcttgccgat

SEQ ID NO: 36 - DNA, 30 bp, Artificial Sequence
  primer
atcggcaagacgggtaagaccggcaagcgc

SEQ ID NO: 37 - DNA, 30 bp, Artificial Sequence
  primer
gcgcttgccggtcttacccgtcttgccgat

SEQ ID NO: 38 - DNA, 30 bp, Artificial Sequence
  primer
atcggcaagacgcagaagaccggcaagcgc

SEQ ID NO: 39 - DNA, 30 bp, Artificial Sequence
  primer
gcgcttgccggtcttctgcgtcttgccgat

SEQ ID NO: 40 - DNA, 30 bp, Artificial Sequence
  primer
gagaagaccggcgctcgctccaccagcgcc

SEQ ID NO: 41 - DNA, 30 bp, Artificial Sequence
  primer
ggcgctggtggagcgagcgccggtcttctc

SEQ ID NO: 42 - DNA, 30 bp, Artificial Sequence
  primer
gagaagaccggcagacgctccaccagcgcc

SEQ ID NO: 43 - DNA, 30 bp, Artificial Sequence
  primer
ggcgctggtggagcgtctgccggtcttctc

SEQ ID NO: 44 - DNA, 30 bp, Artificial Sequence
  primer
gagaagaccggcgaacgctccaccagcgcc

SEQ ID NO: 45 - DNA, 30 bp, Artificial Sequence
  primer
ggcgctggtggagcgttcgccggtcttctc

SEQ ID NO: 46 - DNA, 30 bp, Artificial Sequence
  primer
gagaagaccggctctcgctccaccagcgcc

SEQ ID NO: 47 - DNA, 30 bp, Artificial Sequence
  primer
ggcgctggtggagcgagagccggtcttctc

SEQ ID NO: 48 - DNA, 30 bp, Artificial Sequence
  primer
gagaagaccggcggtcgctccaccagcgcc

SEQ ID NO: 49 - DNA, 30 bp, Artificial Sequence
  primer
ggcgctggtggagcgaccgccggtcttctc

SEQ ID NO: 50 - DNA, 30 bp, Artificial Sequence
  primer
gagaagaccggcgttcgctccaccagcgcc

SEQ ID NO: 51 - DNA, 30 bp, Artificial Sequence
  primer
ggcgctggtggagcgaacgccggtcttctc

SEQ ID NO: 52 - DNA, 30 bp, Artificial Sequence
  primer
gagaagaccggcattcgctccaccagcgcc

SEQ ID NO: 53 - DNA, 30 bp, Artificial Sequence
  primer
ggcgctggtggagcgaatgccggtcttctc

SEQ ID NO: 54 - DNA, 30 bp, Artificial Sequence
  primer
gagaagaccggccttcgctccaccagcgcc

SEQ ID NO: 55 - DNA, 30 bp, Artificial Sequence
  primer
ggcgctggtggagcgaaggccggtcttctc

SEQ ID NO: 56 - DNA, 30 bp, Artificial Sequence
  primer
gagaagaccggcatgcgctccaccagcgcc

SEQ ID NO: 57 - DNA, 30 bp, Artificial Sequence
  primer
ggcgctggtggagcgcatgccggtcttctc

SEQ ID NO: 58 - DNA, 30 bp, Artificial Sequence
  primer
gagaagaccggcttccgctccaccagcgcc

SEQ ID NO: 59 - DNA, 30 bp, Artificial Sequence
  primer
ggcgctggtggagcggaagccggtcttctc

SEQ ID NO: 60 - DNA, 30 bp, Artificial Sequence
  primer
gagaagaccggctatcgctccaccagcgcc

SEQ ID NO: 61 - DNA, 30 bp, Artificial Sequence
  primer
ggcgctggtggagcgatagccggtcttctc

SEQ ID NO: 62 - DNA, 30 bp, Artificial Sequence
  primer
gagaagaccggctggcgctccaccagcgcc

SEQ ID NO: 63 - DNA, 30 bp, Artificial Sequence
  primer
ggcgctggtggagcgccagccggtcttctc

SEQ ID NO: 64 - DNA, 30 bp, Artificial Sequence
  primer
aagaccggcaaggcctccaccagcgccgcc

SEQ ID NO: 65 - DNA, 30 bp, Artificial Sequence
  primer
ggcggcgctggtggaggccttgccggtctt

SEQ ID NO: 66 - DNA, 30 bp, Artificial Sequence
  primer
aagaccggcaaggaatccaccagcgccgcc

SEQ ID NO: 67 - DNA, 30 bp, Artificial Sequence
  primer
ggcggcgctggtggattccttgccggtctt

SEQ ID NO: 68 - DNA, 30 bp, Artificial Sequence
  primer
aagaccggcaagtcttccaccagcgccgcc

SEQ ID NO: 69 - DNA, 30 bp, Artificial Sequence
  primer
ggcggcgctggtggaagacttgccggtctt

SEQ ID NO: 70 - DNA, 30 bp, Artificial Sequence
  primer
aagaccggcaagggttccaccagcgccgcc

SEQ ID NO: 71 - DNA, 30 bp, Artificial Sequence
  primer
ggcggcgctggtggaacccttgccggtctt

SEQ ID NO: 72 - DNA, 30 bp, Artificial Sequence
  primer
aagaccggcaagaagtccaccagcgccgcc

SEQ ID NO: 73 - DNA, 30 bp, Artificial Sequence
  primer
ggcggcgctggtggacttcttgccggtctt

SEQ ID NO: 74 - DNA, 30 bp, Artificial Sequence
  primer
aagaccggcaagttctccaccagcgccgcc

SEQ ID NO: 75 - DNA, 30 bp, Artificial Sequence
  primer
ggcggcgctggtggagaacttgccggtctt

SEQ ID NO: 76 - DNA, 30 bp, Artificial Sequence
  primer
aagaccggcaagatttccaccagcgccgcc

SEQ ID NO: 77 - DNA, 30 bp, Artificial Sequence
  primer
ggcggcgctggtggaaatcttgccggtctt

SEQ ID NO: 78 - DNA, 30 bp, Artificial Sequence
  primer
aagaccggcaagctttccaccagcgccgcc

SEQ ID NO: 79 - DNA, 30 bp, Artificial Sequence
  primer
ggcggcgctggtggaaagcttgccggtctt

SEQ ID NO: 80 - DNA, 30 bp, Artificial Sequence
  primer
aagaccggcaagatgtccaccagcgccgcc

SEQ ID NO: 81 - DNA, 30 bp, Artificial Sequence
  primer
ggcggcgctggtggacatcttgccggtctt

SEQ ID NO: 82 - DNA, 30 bp, Artificial Sequence
  primer
aagaccggcaaggtttccaccagcgccgcc

SEQ ID NO: 83 - DNA, 30 bp, Artificial Sequence
  primer
ggcggcgctggtggaaaccttgccggtctt

SEQ ID NO: 84 - DNA, 30 bp, Artificial Sequence
  primer
aagaccggcaagtggtccaccagcgccgcc

SEQ ID NO: 85 - DNA, 30 bp, Artificial Sequence
  primer
ggcggcgctggtggaccacttgccggtctt

SEQ ID NO: 86 - DNA, 30 bp, Artificial Sequence
  primer
aagaccggcaagtattccaccagcgccgcc

SEQ ID NO: 87 - DNA, 30 bp, Artificial Sequence
  primer
ggcggcgctggtggaatacttgccggtctt

SEQ ID NO: 88 - DNA, 30 bp, Artificial Sequence
  primer
aagaccggcaagcactccaccagcgccgcc

SEQ ID NO: 89 - DNA, 30 bp, Artificial Sequence
  primer
ggcggcgctggtggagtgcttgccggtctt

SEQ ID NO: 90 - DNA, 30 bp, Artificial Sequence
  primer
gtgcgggcctggcttgagaagaccctggag

SEQ ID NO: 91 - DNA, 30 bp, Artificial Sequence
  primer
ctccagggtcttctcaagccaggcccgcac

SEQ ID NO: 92 - DNA, 30 bp, Artificial Sequence
  primer
cgggcctggattaagaagaccctggaggag

SEQ ID NO: 93 - DNA, 30 bp, Artificial Sequence
  primer
ctcctccagggtcttcttaatccaggcccg

SEQ ID NO: 94 - DNA, 24 bp, Artificial Sequence
  primer
gggacccactccatcgagatttct

SEQ ID NO: 95 - DNA, 27 bp, Artificial Sequence
  primer
aactcttcataatgcttgctctgatag

SEQ ID NO: 96 - DNA, 19 bp, Artificial Sequence
  probe
ctgtgaggtcttcatgaag

SEQ ID NO: 97 - DNA, 21 bp, Artificial Sequence
  primer
agccgaagggcatgagctgca

SEQ ID NO: 98 - DNA, 21 bp, Artificial Sequence
  primer
agccgaagggcatgagctaca

SEQ ID NO: 99 - DNA, 24 bp, Artificial Sequence
  primer
agtgtggacaacccccacgtgtgc

SEQ ID NO: 100 - DNA, 20 bp, Artificial Sequence
  probe
cggtggaggtgaggcagatg